European Patent Specification EP 3 806 903 B1, published February 14, 2024. Title: CD79A CHIMERIC ANTIGEN RECEPTORS. Applicant: bluebird bio, Inc. Friedman, Kevin Perkins, Molly Reed. The sequence listing filed with the application follows.

SEQUENCE LISTING (79 sequences)

SEQ ID NO: 1 - protein, 16 aa, Artificial Sequence
  Made in Lab - Light chain CDR1
RSSQSIVHSNGNTYLE

SEQ ID NO: 2 - protein, 7 aa, Artificial Sequence
  Made in Lab - Light chain CDR2
KVSNRFS

SEQ ID NO: 3 - protein, 9 aa, Artificial Sequence
  Made in Lab - Light Chain CDR3
FQGSHVPFT

SEQ ID NO: 4 - protein, 10 aa, Artificial Sequence
  Made in Lab - Heavy chain CDR1
GYTFSTSWMN

SEQ ID NO: 5 - protein, 17 aa, Artificial Sequence
  Made in Lab - Heavy chain CDR2
RIYPGDGDTNYNGKFKG

SEQ ID NO: 6 - protein, 11 aa, Artificial Sequence
  Made in Lab - Heavy chain CDR6
FYYGNTFAMDY

SEQ ID NO: 7 - protein, 112 aa, Artificial Sequence
  Made in Lab - Varialble light chain
DVLMTQIPLSLPVSLGDQASISCRSSQSIVHSNGNTYLEWYLQKPGQSPKLLIYKVSNRFSGVPDRFSGSGSGTDFTLKISRVEAEDLGVYYCFQGSHVPFTFGSGTKLEIK

SEQ ID NO: 8 - protein, 120 aa, Artificial Sequence
  Made in Lab - Variable heavy chain
QVQLQQSGPELVKPGASVKISCKASGYTFSTSWMNWVKQRPGQGLEWIGRIYPGDGDTNYNGKFKGKATLTADKSSNTAYMQLSSLTSVDSAVYFCERFYYGNTFAMDYWGQGTSVTVSS

SEQ ID NO: 9 - protein, 16 aa, Artificial Sequence
  Made in Lab - Light chain CDR1
RSSQSLVHSNGNTYLH

SEQ ID NO: 10 - protein, 7 aa, Artificial Sequence
  Made in Lab - Light chain CDR2
KVSNRFS

SEQ ID NO: 11 - protein, 10 aa, Artificial Sequence
  Made in Lab - Light Chain CDR3
SQSTHVPPYT

SEQ ID NO: 12 - protein, 10 aa, Artificial Sequence
  Made in Lab - Heavy chain CDR1
GYAFSFSWMN

SEQ ID NO: 13 - protein, 17 aa, Artificial Sequence
  Made in Lab - Heavy chain CDR2
RIYPGNGDTNYNGKFKG

SEQ ID NO: 14 - protein, 12 aa, Artificial Sequence
  Made in Lab - Heavy chain CDR6
WVYSGNNYAVDY

SEQ ID NO: 15 - protein, 113 aa, Artificial Sequence
  Made in Lab - Varialble light chain
DVVMTQTPLSLPVSLGDQASISCRSSQSLVHSNGNTYLHWYLQKPGQSPKLLIYKVSNRFSGVPDRFSGSGSGTDFTLKISRVEAEDLGVYFCSQSTHVPPYTFGGGTKLEIK

SEQ ID NO: 16 - protein, 121 aa, Artificial Sequence
  Made in Lab - Variable heavy chain
QVQLQQSGPELVKPGASVKISCKTSGYAFSFSWMNWVKWGPGQGLEWIGRIYPGNGDTNYNGKFKGKATLTADKSSNTAYMQLSSLTSVDSAVYFCARWVYSGNNYAVDYWGQGTSVTVSS

SEQ ID NO: 17 - protein, 14 aa, Artificial Sequence
  Made in Lab - Light chain CDR1
TGTSSDFGSYNLVS

SEQ ID NO: 18 - protein, 7 aa, Artificial Sequence
  Made in Lab - Light chain CDR2
EGSKRPS

SEQ ID NO: 19 - protein, 10 aa, Artificial Sequence
  Made in Lab - Light Chain CDR3
CSYAGGSTWV

SEQ ID NO: 20 - protein, 10 aa, Artificial Sequence
  Made in Lab - Heavy chain CDR1
GLTFTSYAMN

SEQ ID NO: 21 - protein, 17 aa, Artificial Sequence
  Made in Lab - Heavy chain CDR2
GISGSGGGTYYADSVKG

SEQ ID NO: 22 - protein, 7 aa, Artificial Sequence
  Made in Lab - Heavy chain CDR6
LGGWSDY

SEQ ID NO: 23 - protein, 110 aa, Artificial Sequence
  Made in Lab - Varialble light chain
QSALTQPASVSGSPGQSITISCTGTSSDFGSYNLVSWYQQHPGKAPKLMIYEGSKRPSGVSNRFSGSKSGNTASLTISGLQAEDEADYYCCSYAGGSTWVFGGGTKLTVL

SEQ ID NO: 24 - protein, 116 aa, Artificial Sequence
  Made in Lab - Variable heavy chain
EVQLLESGGGLVQPGGSLRLSCAASGLTFTSYAMNWVRQAPGKGLEWVSGISGSGGGTYYADSVKGRFTISRDNSKNTLYLQMNSLRAEDTAVYYCAKLGGWSDYWGQGTLVTVSS

SEQ ID NO: 25 - protein, 492 aa, Artificial Sequence
  Made in Lab - anti-CD79A-01_HL CAR construct
MALPVTALLLPLALLLHAARPQVQLQQSGPELVKPGASVKISCKASGYTFSTSWMNWVKQRPGQGLEWIGRIYPGDGDTNYNGKFKGKATLTADKSSNTAYMQLSSLTSVDSAVYFCERFYYGNTFAMDYWGQGTSVTVSSGGGGSGGGGSGGGGSDVLMTQIPLSLPVSLGDQASISCRSSQSIVHSNGNTYLEWYLQKPGQSPKLLIYKVSNRFSGVPDRFSGSGSGTDFTLKISRVEAEDLGVYYCFQGSHVPFTFGSGTKLEIKRTTTPAPRPPTPAPTIASQPLSLRPEACRPAAGGAVHTRGLDFACDIYIWAPLAGTCGVLLLSLVITLYCKRGRKKLLYIFKQPFMRPVQTTQEEDGCSCRFPEEEEGGCELRVKFSRSADAPAYQQGQNQLYNELNLGRREEYDVLDKRRGRDPEMGGKPRRKNPQEGLYNELQKDKMAEAYSEIGMKGERRRGKGHDGLYQGLSTATKDTYDALHMQALPPR

SEQ ID NO: 26 - protein, 492 aa, Artificial Sequence
  Made in Lab - anti-CD79A-01_LH CAR construct
MALPVTALLLPLALLLHAARPDVLMTQIPLSLPVSLGDQASISCRSSQSIVHSNGNTYLEWYLQKPGQSPKLLIYKVSNRFSGVPDRFSGSGSGTDFTLKISRVEAEDLGVYYCFQGSHVPFTFGSGTKLEIKRGGGGSGGGGSGGGGSQVQLQQSGPELVKPGASVKISCKASGYTFSTSWMNWVKQRPGQGLEWIGRIYPGDGDTNYNGKFKGKATLTADKSSNTAYMQLSSLTSVDSAVYFCERFYYGNTFAMDYWGQGTSVTVSSTTTPAPRPPTPAPTIASQPLSLRPEACRPAAGGAVHTRGLDFACDIYIWAPLAGTCGVLLLSLVITLYCKRGRKKLLYIFKQPFMRPVQTTQEEDGCSCRFPEEEEGGCELRVKFSRSADAPAYQQGQNQLYNELNLGRREEYDVLDKRRGRDPEMGGKPRRKNPQEGLYNELQKDKMAEAYSEIGMKGERRRGKGHDGLYQGLSTATKDTYDALHMQALPPR

SEQ ID NO: 27 - protein, 493 aa, Artificial Sequence
  Made in Lab - anti-CD79A-10_HL CAR construct
MALPVTALLLPLALLLHAARPQVQLQQSGPELVKPGASVKISCKTSGYAFSFSWMNWVKWGPGQGLEWIGRIYPGNGDTNYNGKFKGKATLTADKSSNTAYMQLSSLTSVDSAVYFCARWVYSGNNYAVDYWGQGTSVTVSSGGGGSGGGGSGGGGSDVVMTQTPLSLPVSLGDQASISCRSSQSLVHSNGNTYLHWYLQKPGQSPKLLIYKVSNRFSGVPDRFSGSGSGTDFTLKISRVEAEDLGVYFCSQSTHVPPYTFGGGTKLEIKTTTPAPRPPTPAPTIASQPLSLRPEACRPAAGGAVHTRGLDFACDIYIWAPLAGTCGVLLLSLVITLYCKRGRKKLLYIFKQPFMRPVQTTQEEDGCSCRFPEEEEGGCELRVKFSRSADAPAYQQGQNQLYNELNLGRREEYDVLDKRRGRDPEMGGKPRRKNPQEGLYNELQKDKMAEAYSEIGMKGERRRGKGHDGLYQGLSTATKDTYDALHMQALPPR

SEQ ID NO: 28 - protein, 493 aa, Artificial Sequence
  Made in Lab - anti-CD79A-10_LH CAR construct
MALPVTALLLPLALLLHAARPDVVMTQTPLSLPVSLGDQASISCRSSQSLVHSNGNTYLHWYLQKPGQSPKLLIYKVSNRFSGVPDRFSGSGSGTDFTLKISRVEAEDLGVYFCSQSTHVPPYTFGGGTKLEIKGGGGSGGGGSGGGGSQVQLQQSGPELVKPGASVKISCKTSGYAFSFSWMNWVKWGPGQGLEWIGRIYPGNGDTNYNGKFKGKATLTADKSSNTAYMQLSSLTSVDSAVYFCARWVYSGNNYAVDYWGQGTSVTVSSTTTPAPRPPTPAPTIASQPLSLRPEACRPAAGGAVHTRGLDFACDIYIWAPLAGTCGVLLLSLVITLYCKRGRKKLLYIFKQPFMRPVQTTQEEDGCSCRFPEEEEGGCELRVKFSRSADAPAYQQGQNQLYNELNLGRREEYDVLDKRRGRDPEMGGKPRRKNPQEGLYNELQKDKMAEAYSEIGMKGERRRGKGHDGLYQGLSTATKDTYDALHMQALPPR

SEQ ID NO: 29 - protein, 485 aa, Artificial Sequence
  Made in Lab - anti-CD79A-02_HL CAR construct
MALPVTALLLPLALLLHAARPEVQLLESGGGLVQPGGSLRLSCAASGLTFTSYAMNWVRQAPGKGLEWVSGISGSGGGTYYADSVKGRFTISRDNSKNTLYLQMNSLRAEDTAVYYCAKLGGWSDYWGQGTLVTVSSGGGGSGGGGSGGGGSQSALTQPASVSGSPGQSITISCTGTSSDFGSYNLVSWYQQHPGKAPKLMIYEGSKRPSGVSNRFSGSKSGNTASLTISGLQAEDEADYYCCSYAGGSTWVFGGGTKLTVLTTTPAPRPPTPAPTIASQPLSLRPEACRPAAGGAVHTRGLDFACDIYIWAPLAGTCGVLLLSLVITLYCKRGRKKLLYIFKQPFMRPVQTTQEEDGCSCRFPEEEEGGCELRVKFSRSADAPAYQQGQNQLYNELNLGRREEYDVLDKRRGRDPEMGGKPRRKNPQEGLYNELQKDKMAEAYSEIGMKGERRRGKGHDGLYQGLSTATKDTYDALHMQALPPR

SEQ ID NO: 30 - protein, 485 aa, Artificial Sequence
  Made in Lab - anti-CD79A-02_LH CAR construct
MALPVTALLLPLALLLHAARPQSALTQPASVSGSPGQSITISCTGTSSDFGSYNLVSWYQQHPGKAPKLMIYEGSKRPSGVSNRFSGSKSGNTASLTISGLQAEDEADYYCCSYAGGSTWVFGGGTKLTVLGGGGSGGGGSGGGGSEVQLLESGGGLVQPGGSLRLSCAASGLTFTSYAMNWVRQAPGKGLEWVSGISGSGGGTYYADSVKGRFTISRDNSKNTLYLQMNSLRAEDTAVYYCAKLGGWSDYWGQGTLVTVSSTTTPAPRPPTPAPTIASQPLSLRPEACRPAAGGAVHTRGLDFACDIYIWAPLAGTCGVLLLSLVITLYCKRGRKKLLYIFKQPFMRPVQTTQEEDGCSCRFPEEEEGGCELRVKFSRSADAPAYQQGQNQLYNELNLGRREEYDVLDKRRGRDPEMGGKPRRKNPQEGLYNELQKDKMAEAYSEIGMKGERRRGKGHDGLYQGLSTATKDTYDALHMQALPPR

SEQ ID NO: 31 - DNA, 1479 bp, Artificial Sequence
  Made in Lab - anti-CD79A-01_HL CAR polynucleotide construct
atggcacttccagtgactgcattgttgttgcccctggccctgctgcttcacgccgcaaggccccaggtccagcttcagcagtccggaccagagttggtgaaacctggggcatcagtcaagattagctgcaaggcatcagggtacaccttcagcactagttggatgaattgggtgaagcagcggcctggccaggggttggagtggatcggacgcatctacccaggggatggcgatacaaactacaacggaaagtttaaaggtaaggctactttgaccgctgacaaatcatcaaacacggcatatatgcaactgtctagcctcacatctgtcgactctgccgtctacttttgcgagcgattctactatggcaacacttttgccatggactactgggggcaggggacatcagtaacagttagttctggagggggcggttccgggggcgggggatccggagggggaggcagtgatgtgctgatgacccagataccgttgtcactcccggtctcactgggtgaccaggcaagcatcagctgcaggagcagccagtccatcgtgcactctaacggaaatacctacctggagtggtatctgcagaaacctggccagtcccctaagttgttgatttacaaagtttcaaaccgatttagtggagttcccgataggttttccggttccgggagcggtacagacttcaccctgaagataagtcgggttgaggctgaagacctgggagtatattattgctttcagggcagccacgtaccattcacatttgggagtggaaccaaactggagatcaaaagaaccacaacacctgctccaaggccccccacacccgctccaactatagccagccaaccattgagcctcagacctgaagcttgcaggcccgcagcaggaggcgccgtccatacgcgaggcctggacttcgcgtgtgatatttatatttgggcccctttggccggaacatgtggggtgttgcttctctcccttgtgatcactctgtattgtaagcgcgggagaaagaagctcctgtacatcttcaagcagccttttatgcgacctgtgcaaaccactcaggaagaagatgggtgttcatgccgcttccccgaggaggaagaaggagggtgtgaactgagggtgaaattttctagaagcgccgatgctcccgcatatcagcagggtcagaatcagctctacaatgaattgaatctcggcaggcgagaagagtacgatgttctggacaagagacggggcagggatcccgagatggggggaaagccccggagaaaaaatcctcaggaggggttgtacaatgagctgcagaaggacaagatggctgaagcctatagcgagatcggaatgaaaggcgaaagacgcagaggcaaggggcatgacggtctgtaccagggtctctctacagccaccaaggacacttatgatgcgttgcatatgcaagccttgccaccccgctaa

SEQ ID NO: 32 - DNA, 1479 bp, Artificial Sequence
  Made in Lab - anti-CD79A-01_LH CAR polynucleotide construct
atggctctgcctgtgacggccctgcttttgcccctcgccctgcttctgcatgccgcgagacccgacgtgttgatgacccaaataccgcttagtctgcctgtatctcttggggaccaggctagcatctcatgccgcagcagtcaatccattgtgcactcaaatgggaacacctatttggagtggtatctgcaaaaaccgggacagtctccgaaactgctgatatacaaagtaagcaacaggttcagcggagttcctgacagattcagcggaagcggttctggaactgactttacacttaagatctctcgcgttgaggcggaggacctgggcgtgtattactgttttcaaggatcccacgtcccgtttacattcggatcaggcaccaagctggagatcaagcgcggtggcgggggttctggcgggggcggatccggaggcggcggatcccaggtgcagctgcagcagtctggaccagaactggttaagcccggagcttcagttaagatttcctgtaaggcttcaggctatacattttccacttcttggatgaactgggtgaaacagcgccctggccaggggctggaatggatcggacggatctatcccggcgatggagacactaattataacggtaagttcaaagggaaggccaccctcacggccgacaagtcctccaatacagcgtacatgcaactcagttccctgaccagcgttgatagcgcagtttacttctgtgagcgcttctattacggaaacaccttcgctatggattactggggtcaggggacctccgtgaccgtgtcctctaccacaacacctgctccaaggccccccacacccgctccaactatagccagccaaccattgagcctcagacctgaagcttgcaggcccgcagcaggaggcgccgtccatacgcgaggcctggacttcgcgtgtgatatttatatttgggcccctttggccggaacatgtggggtgttgcttctctcccttgtgatcactctgtattgtaagcgcgggagaaagaagctcctgtacatcttcaagcagccttttatgcgacctgtgcaaaccactcaggaagaagatgggtgttcatgccgcttccccgaggaggaagaaggagggtgtgaactgagggtgaaattttctagaagcgccgatgctcccgcatatcagcagggtcagaatcagctctacaatgaattgaatctcggcaggcgagaagagtacgatgttctggacaagagacggggcagggatcccgagatggggggaaagccccggagaaaaaatcctcaggaggggttgtacaatgagctgcagaaggacaagatggctgaagcctatagcgagatcggaatgaaaggcgaaagacgcagaggcaaggggcatgacggtctgtaccagggtctctctacagccaccaaggacacttatgatgcgttgcatatgcaagccttgccaccccgctaa

SEQ ID NO: 33 - DNA, 1482 bp, Artificial Sequence
  Made in Lab - anti-CD79A-10_HL CAR polynucleotide construct
atggctctgccagtgactgcgctgctgctgcccctcgctcttctgctgcacgccgctcggccacaggtccaactgcaacagagcggccccgagctggtaaaacccggggcctccgtaaaaatatcctgcaagaccagcggctatgccttttcattctcctggatgaactgggtgaagtggggacccggtcagggacttgagtggatcgggcgaatctatcccggaaacggggacacgaattacaacggcaaatttaaaggcaaggctactctgactgctgacaaaagtagcaacaccgcctacatgcagttgtcctctttgacatcagtagactctgcagtgtatttttgcgcccggtgggtttactccggaaataactacgcggttgactattggggacagggcacctccgtgacagtgtcttctggcggcgggggatcaggtggcggcgggtctgggggtggagggagcgacgtggttatgacccagacccctttgagcctgcccgtgagccttggcgaccaagcctccatctcttgccggtcctctcaatcactggtgcacagtaacgggaatacttatctccactggtatttgcaaaagcccggtcagtctcctaagcttctgatctataaggtgtccaaccgcttttctggagtgcccgatagattttccggatctggatccggaacagacttcacattgaagattagtagagtcgaagcggaggacttgggtgtttatttttgttcccagagtacccacgtgcctccatacacgtttggaggtggaaccaaacttgaaattaagaccacaacacctgctccaaggccccccacacccgctccaactatagccagccaaccattgagcctcagacctgaagcttgcaggcccgcagcaggaggcgccgtccatacgcgaggcctggacttcgcgtgtgatatttatatttgggcccctttggccggaacatgtggggtgttgcttctctcccttgtgatcactctgtattgtaagcgcgggagaaagaagctcctgtacatcttcaagcagccttttatgcgacctgtgcaaaccactcaggaagaagatgggtgttcatgccgcttccccgaggaggaagaaggagggtgtgaactgagggtgaaattttctagaagcgccgatgctcccgcatatcagcagggtcagaatcagctctacaatgaattgaatctcggcaggcgagaagagtacgatgttctggacaagagacggggcagggatcccgagatggggggaaagccccggagaaaaaatcctcaggaggggttgtacaatgagctgcagaaggacaagatggctgaagcctatagcgagatcggaatgaaaggcgaaagacgcagaggcaaggggcatgacggtctgtaccagggtctctctacagccaccaaggacacttatgatgcgttgcatatgcaagccttgccaccccgctaa

SEQ ID NO: 34 - DNA, 1482 bp, Artificial Sequence
  Made in Lab - anti-CD79A-10_LH CAR polynucleotide construct
atggccctgccagtaacagcactgctccttcctctcgcactcctcctgcacgcagcaagaccagatgtcgtgatgactcagacacctcttagcttgcccgtctccttgggtgatcaggctagcatttcatgtagatcaagccagagcttggtacattcaaatggcaatacctacctgcactggtatctccagaaacctggccagagcccaaaattgcttatctataaagttagtaacagattctccggggtcccagatcgattttccggctcaggctcaggcacggattttaccctgaagatctcacgagtcgaggcagaagatcttggcgtgtacttttgttcccagagtacccacgtacccccttacacattcggaggagggaccaagttggagatcaaaggaggggggggcagtggggggggcggttccggagggggaggaagccaagtacaactgcaacaaagcggacccgagctcgtcaaacctggtgctagcgtcaaaatttcctgtaagaccagcggctacgcttttagcttttcttggatgaactgggtgaaatgggggccggggcagggcctggagtggataggacgaatttatcccgggaatggggatacaaattacaatggtaaattcaaggggaaagccacactgactgcagataaaagctccaacacggcatacatgcagctcagctccctcacttctgtggattctgctgtttacttttgtgccaggtgggtttactctggtaataactatgccgtggattactgggggcaaggcacctctgttacagtgagttccaccacaacacctgctccaaggccccccacacccgctccaactatagccagccaaccattgagcctcagacctgaagcttgcaggcccgcagcaggaggcgccgtccatacgcgaggcctggacttcgcgtgtgatatttatatttgggcccctttggccggaacatgtggggtgttgcttctctcccttgtgatcactctgtattgtaagcgcgggagaaagaagctcctgtacatcttcaagcagccttttatgcgacctgtgcaaaccactcaggaagaagatgggtgttcatgccgcttccccgaggaggaagaaggagggtgtgaactgagggtgaaattttctagaagcgccgatgctcccgcatatcagcagggtcagaatcagctctacaatgaattgaatctcggcaggcgagaagagtacgatgttctggacaagagacggggcagggatcccgagatggggggaaagccccggagaaaaaatcctcaggaggggttgtacaatgagctgcagaaggacaagatggctgaagcctatagcgagatcggaatgaaaggcgaaagacgcagaggcaaggggcatgacggtctgtaccagggtctctctacagccaccaaggacacttatgatgcgttgcatatgcaagccttgccaccccgctaa

SEQ ID NO: 35 - DNA, 1458 bp, Artificial Sequence
  Made in Lab - anti-CD79A-02_HL CAR polynucleotide construct
atggcgcttcctgtcactgccctgcttctgcccctcgctcttctgctgcacgccgctcgccccgaagttcagctgttggaaagcggaggcggcctggttcaacccggtggcagtctgaggctgtcctgcgccgcctccggtcttacattcacatcttacgctatgaattgggtgcgccaagcccccggcaagggcctggagtgggttagtggtatcagcgggtccggaggagggacttactacgccgactctgtaaagggacggttcactatctcccgggacaactccaaaaacacactttacctgcagatgaactccttgcgagccgaagacacagccgtgtactactgtgctaagcttggaggctggagtgattattggggtcaggggaccttggtgacagtgtcttccgggggtgggggatccggtggcggtggatcaggagggggtggctcccagagcgctctcacacagccggccagtgtgtcaggatcacctggacagtccattacgatctcttgcactggaacaagctctgactttggctcctataatctcgtgtcctggtatcagcagcaccccgggaaggctcccaagcttatgatttacgagggctcaaaacgcccttcaggtgtatccaaccgattcagcggaagcaaatccggcaataccgcaagtctcaccataagtggcctgcaggcagaagacgaagccgactactattgttgttcttatgccggcggctcaacatgggtgttcggcgggggcaccaagctgactgtattgaccacaacacctgctccaaggccccccacacccgctccaactatagccagccaaccattgagcctcagacctgaagcttgcaggcccgcagcaggaggcgccgtccatacgcgaggcctggacttcgcgtgtgatatttatatttgggcccctttggccggaacatgtggggtgttgcttctctcccttgtgatcactctgtattgtaagcgcgggagaaagaagctcctgtacatcttcaagcagccttttatgcgacctgtgcaaaccactcaggaagaagatgggtgttcatgccgcttccccgaggaggaagaaggagggtgtgaactgagggtgaaattttctagaagcgccgatgctcccgcatatcagcagggtcagaatcagctctacaatgaattgaatctcggcaggcgagaagagtacgatgttctggacaagagacggggcagggatcccgagatggggggaaagccccggagaaaaaatcctcaggaggggttgtacaatgagctgcagaaggacaagatggctgaagcctatagcgagatcggaatgaaaggcgaaagacgcagaggcaaggggcatgacggtctgtaccagggtctctctacagccaccaaggacacttatgatgcgttgcatatgcaagccttgccaccccgctaa

SEQ ID NO: 36 - DNA, 1458 bp, Artificial Sequence
  Made in Lab - anti-CD79A-02_LH CAR polynucleotide construct
atggctctgcctgtaactgctctgctgcttccccttgctctgctcctgcatgccgcccggccgcaaagcgccctgactcagccagcttccgtgtctggctctccggggcagtccatcaccatctcatgcacaggaacctccagcgacttcggatcatataacctggtttcatggtatcagcagcatcctgggaaggctccgaagttgatgatctacgagggaagcaagaggcccagtggggtcagtaaccgcttctctggaagtaagtcaggcaataccgctagtctgaccatctccggattgcaagctgaggacgaagctgattactactgctgttcatatgcagggggttctacttgggtgttcggcggtggaaccaagcttaccgttctgggaggcggaggctccgggggaggcggatcaggcggaggtggatccgaagtgcagctgcttgagtcaggagggggattggtccagccggggggatcattgaggctgtcttgtgccgcaagtggactcacttttaccagttatgcaatgaactgggtgcggcaggcacccgggaagggactggaatgggtgagtggcatatctggcagcgggggcggaacttactacgctgattctgtcaagggaaggtttactatctcacgagacaacagcaaaaacaccctctacctgcagatgaactcactcagagcagaggatactgcagtctactattgtgctaagctgggtggttggagcgactactggggacaagggacgttggtgaccgtgtcttcaaccacaacacctgctccaaggccccccacacccgctccaactatagccagccaaccattgagcctcagacctgaagcttgcaggcccgcagcaggaggcgccgtccatacgcgaggcctggacttcgcgtgtgatatttatatttgggcccctttggccggaacatgtggggtgttgcttctctcccttgtgatcactctgtattgtaagcgcgggagaaagaagctcctgtacatcttcaagcagccttttatgcgacctgtgcaaaccactcaggaagaagatgggtgttcatgccgcttccccgaggaggaagaaggagggtgtgaactgagggtgaaattttctagaagcgccgatgctcccgcatatcagcagggtcagaatcagctctacaatgaattgaatctcggcaggcgagaagagtacgatgttctggacaagagacggggcagggatcccgagatggggggaaagccccggagaaaaaatcctcaggaggggttgtacaatgagctgcagaaggacaagatggctgaagcctatagcgagatcggaatgaaaggcgaaagacgcagaggcaaggggcatgacggtctgtaccagggtctctctacagccaccaaggacacttatgatgcgttgcatatgcaagccttgccaccccgctaa

SEQ ID NO: 37 - protein, 226 aa, Homo sapiens
MPGGPGVLQALPATIFLLFLLSAVYLGPGCQALWMHKVPASLMVSLGEDAHFQCPHNSSNNANVTWWRVLHGNYTWPPEFLGPGEDPNGTLIIQNVNKSHGGIYVCRVQEGNESYQQSCGTYLRVRQPPPRPFLDMGEGTKNRIITAEGIILLFCAVVPGTLLLFRKRWQNEKLGLDAGDEYEDENLYEGLNLDDCSMYEDISRGLQGTYQDVGSLNIGDVQLEKP

SEQ ID NO: 38 - protein, 188 aa, Homo sapiens
MPGGPGVLQALPATIFLLFLLSAVYLGPGCQALWMHKVPASLMVSLGEDAHFQCPHNSSNNANVTWWRVLHGNYTWPPEFLGPGEDPNEPPPRPFLDMGEGTKNRIITAEGIILLFCAVVPGTLLLFRKRWQNEKLGLDAGDEYEDENLYEGLNLDDCSMYEDISRGLQGTYQDVGSLNIGDVQLEKP

SEQ ID NO: 39 - protein, 5 aa, Artificial Sequence
  Exemplary linker sequence
DGGGS

SEQ ID NO: 40 - protein, 5 aa, Artificial Sequence
  Exemplary linker sequence
TGEKP

SEQ ID NO: 41 - protein, 4 aa, Artificial Sequence
  Exemplary linker sequence
GGRR

SEQ ID NO: 42 - protein, 5 aa, Artificial Sequence
  Exemplary linker sequence
GGGGS

SEQ ID NO: 43 - protein, 14 aa, Artificial Sequence
  Exemplary linker sequence
EGKSSGSGSESKVD

SEQ ID NO: 44 - protein, 18 aa, Artificial Sequence
  Exemplary linker sequence
KESGSVSSEQLAQFRSLD

SEQ ID NO: 45 - protein, 8 aa, Artificial Sequence
  Exemplary linker sequence
GGRRGGGS

SEQ ID NO: 46 - protein, 9 aa, Artificial Sequence
  Exemplary linker sequence
LRQRDGERP

SEQ ID NO: 47 - protein, 12 aa, Artificial Sequence
  Exemplary linker sequence
LRQKDGGGSERP

SEQ ID NO: 48 - protein, 16 aa, Artificial Sequence
  Exemplary linker sequence
LRQKDGGGSGGGSERP

SEQ ID NO: 49 - protein, 18 aa, Artificial Sequence
  Exemplary linker sequence
GSTSGSGKPGSGEGSTKG

SEQ ID NO: 50 - protein, 7 aa, Artificial Sequence
  Cleavage sequence by TEV protease
  misc_feature (2)..(3): Xaa is any amino acid
  misc_feature (5)..(5): Xaa is any amino acid
  MISC_FEATURE (7)..(7): Xaa = Gly or Ser
EXXYXQX

SEQ ID NO: 51 - protein, 7 aa, Artificial Sequence
  Cleavage sequence by TEV protease
ENLYFQG

SEQ ID NO: 52 - protein, 7 aa, Artificial Sequence
  Cleavage sequence by TEV protease
ENLYFQS

SEQ ID NO: 53 - protein, 22 aa, Artificial Sequence
  Self-cleaving polypeptide comprising 2A site
GSGATNFSLLKQAGDVEENPGP

SEQ ID NO: 54 - protein, 19 aa, Artificial Sequence
  Self-cleaving polypeptide comprising 2A site
ATNFSLLKQAGDVEENPGP

SEQ ID NO: 55 - protein, 14 aa, Artificial Sequence
  Self-cleaving polypeptide comprising 2A site
LLKQAGDVEENPGP

SEQ ID NO: 56 - protein, 21 aa, Artificial Sequence
  Self-cleaving polypeptide comprising 2A site
GSGEGRGSLLTCGDVEENPGP

SEQ ID NO: 57 - protein, 18 aa, Artificial Sequence
  Self-cleaving polypeptide comprising 2A site
EGRGSLLTCGDVEENPGP

SEQ ID NO: 58 - protein, 13 aa, Artificial Sequence
  Self-cleaving polypeptide comprising 2A site
LLTCGDVEENPGP

SEQ ID NO: 59 - protein, 23 aa, Artificial Sequence
  Self-cleaving polypeptide comprising 2A site
GSGQCTNYALLKLAGDVESNPGP

SEQ ID NO: 60 - protein, 20 aa, Artificial Sequence
  Self-cleaving polypeptide comprising 2A site
QCTNYALLKLAGDVESNPGP

SEQ ID NO: 61 - protein, 14 aa, Artificial Sequence
  Self-cleaving polypeptide comprising 2A site
LLKLAGDVESNPGP

SEQ ID NO: 62 - protein, 25 aa, Artificial Sequence
  Self-cleaving polypeptide comprising 2A site
GSGVKQTLNFDLLKLAGDVESNPGP

SEQ ID NO: 63 - protein, 22 aa, Artificial Sequence
  Self-cleaving polypeptide comprising 2A site
VKQTLNFDLLKLAGDVESNPGP

SEQ ID NO: 64 - protein, 14 aa, Artificial Sequence
  Self-cleaving polypeptide comprising 2A site
LLKLAGDVESNPGP

SEQ ID NO: 65 - protein, 19 aa, Artificial Sequence
  Self-cleaving polypeptide comprising 2A site
LLNFDLLKLAGDVESNPGP

SEQ ID NO: 66 - protein, 19 aa, Artificial Sequence
  Self-cleaving polypeptide comprising 2A site
TLNFDLLKLAGDVESNPGP

SEQ ID NO: 67 - protein, 14 aa, Artificial Sequence
  Self-cleaving polypeptide comprising 2A site
LLKLAGDVESNPGP

SEQ ID NO: 68 - protein, 17 aa, Artificial Sequence
  Self-cleaving polypeptide comprising 2A site
NFDLLKLAGDVESNPGP

SEQ ID NO: 69 - protein, 20 aa, Artificial Sequence
  Self-cleaving polypeptide comprising 2A site
QLLNFDLLKLAGDVESNPGP

SEQ ID NO: 70 - protein, 24 aa, Artificial Sequence
  Self-cleaving polypeptide comprising 2A site
APVKQTLNFDLLKLAGDVESNPGP

SEQ ID NO: 71 - protein, 40 aa, Artificial Sequence
  Self-cleaving polypeptide comprising 2A site
VTELLYRMKRAETYCPRPLLAIHPTEARHKQKIVAPVKQT

SEQ ID NO: 72 - protein, 18 aa, Artificial Sequence
  Self-cleaving polypeptide comprising 2A site
LNFDLLKLAGDVESNPGP

SEQ ID NO: 73 - protein, 40 aa, Artificial Sequence
  Self-cleaving polypeptide comprising 2A site
LLAIHPTEARHKQKIVAPVKQTLNFDLLKLAGDVESNPGP

SEQ ID NO: 74 - protein, 33 aa, Artificial Sequence
  Self-cleaving polypeptide comprising 2A site
EARHKQKIVAPVKQTLNFDLLKLAGDVESNPGP

SEQ ID NO: 75 - DNA, 10 bp, Artificial Sequence
  Consensus Kozak sequence
gccrccatgg

SEQ ID NO: 76 - protein, 4 aa, Artificial Sequence
  Exemplary rule for determining light chain CDR-L3 motif
  MISC_FEATURE (3)..(3): Xaa is any amino acid
FGXG

SEQ ID NO: 77 - protein, 4 aa, Artificial Sequence
  Exemplary rule for determining heavy chain CDR-H1motif
  MISC_FEATURE (2)..(4): Xaa is any amino acid
CXXX

SEQ ID NO: 78 - protein, 5 aa, Artificial Sequence
  Exemplary rule for determining heavy chain CDR-H2motif
LEWIG

SEQ ID NO: 79 - protein, 4 aa, Artificial Sequence
  Exemplary rule for determining heavy chain CDR-H3 motif
  MISC_FEATURE (3)..(3): Xaa is any amino acid
WGXG